European Patent Specification EP 3 619 313 B9, published October 4, 2023. Title: TUMOR ENVIRONMENT SPECIFIC EXPRESSION OF CHIMERIC ANTIGEN. Applicant: The National Institute for Biotechnology in the Negev Ltd. The sequence listing filed with the application follows.

SEQUENCE LISTING (47 sequences)

SEQ ID NO: 1 - DNA, 9 bp, Homo sapiens
ttccgggaa

SEQ ID NO: 2 - DNA, 10 bp, Homo sapiens
gggaatttcc

SEQ ID NO: 3 - DNA, 31 bp, Homo sapiens
gaccttgagtacgtgcgtctctgcacgtatg

SEQ ID NO: 4 - DNA, 26 bp, Homo sapiens
gcgcttcctgacagtgacgcgagccg

SEQ ID NO: 5 - DNA, 126 bp, ARTIFICIAL SEQUENCE
  SYNTHETIC PROMOTER
gggaatttccggggactttccgggaatttccggggactttccgggaatttccagagcatattaaggtgacgcgtgtggcctcgaacaccgagcgaccctgcagcgacccgcttaaaagcggccgcc

SEQ ID NO: 6 - DNA, 163 bp, ARTIFICIAL SEQUENCE
  SYNTHETIC PROMOTER
ttccgggaaagggtgggcaagtttccgggaaagcagtaggtacagccttccgggaaagggtgggcaagtttccgggaaagcagtaggtttttcgcatattaaggtgacgcgtgtggcctcgaacaccgagcgaccctgcagcgacccgcttaaaaggcgcgcc

SEQ ID NO: 7 - DNA, 257 bp, ARTIFICIAL SEQUENCE
  SYNTHETIC PROMOTER
ttccgggaaagggtgggcaagtttccgggaaagcagtaggtacagccttccgggaaagggtgggcaagtttccgggaaagcagtaggtacagccttccgggaaagggtgggcaagtttccgggaaagcagtaggtacagccttccgggaaagggtgggcaagtttccgggaaagcagtaggtttttcgcatattaaggtgacgcgtgtggcctcgaacaccgagcgaccctgcagcgacccgcttaaaaggcgcgcc

SEQ ID NO: 8 - DNA, 351 bp, ARTIFICIAL SEQUENCE
  SYNTHETIC PROMOTER
ttccgggaaagggtgggcaagtttccgggaaagcagtaggtacagccttccgggaaagggtgggcaagtttccgggaaagcagtaggtacagccttccgggaaagggtgggcaagtttccgggaaagcagtaggtacagccttccgggaaagggtgggcaagtttccgggaaagcagtaggtacagccttccgggaaagggtgggcaagtttccgggaaagcagtaggtacagccttccgggaaagggtgggcaagtttccgggaaagcagtaggtttttcgcatattaaggtgacgcgtgtggcctcgaacaccgagcgaccctgcagcgacccgcttaaaaggcgcgcc

SEQ ID NO: 9 - DNA, 160 bp, ARTIFICIAL SEQUENCE
  SYNTHETIC PROMOTER
ttccgggaaagggtgggcaagtttccgggaacccgggaatttccggggactttccgggaatttccggggactttccgggaatttccagagcatattaaggtgacgcgtgtggcctcgaacaccgagcgaccctgcagcgacccgcttaaaagcggccgcc

SEQ ID NO: 10 - DNA, 139 bp, ARTIFICIAL SEQUENCE
  SYNTHETIC PROMOTER
ttccgggaaagggtgggcaagtttccgggaacccgggaatttccggggactttccgggaatttccagagcatattaaggtgacgcgtgtggcctcgaacaccgagcgaccctgcagcgacccgcttaaaagcggccgcc

SEQ ID NO: 11 - DNA, 267 bp, ARTIFICIAL SEQUENCE
  SYNTHETIC PROMOTER
ttccgggaaagggtgggcaagtttccgggaaagcagtaggtacagccttccgggaaagggtgggcaagtttccgggaaagagcagggaatttccggggactttccgggaatttccggggactttccgggaatttccagagcagggaatttccggggactttccgggaatttccggggactttccgggaatttccagagcatattaaggtgacgcgtgtggcctcgaacaccgagcgaccctgcagcgacccgcttaaaaggcgcgcc

SEQ ID NO: 12 - DNA, 372 bp, ARTIFICIAL SEQUENCE
  SYNTHETIC PROMOTER
ttccgggaaagggtgggcaagtttccgggaaagcagtaggtacagccttccgggaaagggtgggcaagtttccgggaaagcagtaggtacagccttccgggaaagggtgggcaagtttccgggaaagagcagggaatttccggggactttccgggaatttccggggactttccgggaatttccagagcagggaatttccggggactttccgggaatttccggggactttccgggaatttccagagcagggaatttccggggactttccgggaatttccggggactttccgggaatttccagagcatattaaggtgacgcgtgtggcctcgaacaccgagcgaccctgcagcgacccgcttaaaaggcgcgcc

SEQ ID NO: 13 - DNA, 456 bp, ARTIFICIAL SEQUENCE
  SYNTHETIC PROMOTER
ttccgggaaagggtgggcaagtttccgggaaagcagtaggtacagccttccgggaaagggtgggcaagtttccgggaaagcagtaggtacagccttccgggaaagggtgggcaagtttccgggaaagcagtaggtacagccgaccttgagtacgtgcgtctctgcacgtatgagagcagaccttgagtacgtgcgtctctgcacgtatgagagcagggaatttccggggactttccgggaatttccggggactttccgggaatttccagagcagggaatttccggggactttccgggaatttccggggactttccgggaatttccagagcagggaatttccggggactttccgggaatttccggggactttccgggaatttccagagcatattaaggtgacgcgtgtggcctcgaacaccgagcgaccctgcagcgacccgcttaaaaggcgcgcc

SEQ ID NO: 14 - DNA, 446 bp, ARTIFICIAL SEQUENCE
  SYNTHETIC PROMOTER
ttccgggaaagggtgggcaagtttccgggaaagcagtaggtacagccttccgggaaagggtgggcaagtttccgggaaagcagtaggtacagccttccgggaaagggtgggcaagtttccgggaaagagcagggaatttccggggactttccgggaatttccggggactttccgggaatttccagagcagggaatttccggggactttccgggaatttccggggactttccgggaatttccagagcagggaatttccggggactttccgggaatttccggggactttccgggaatttccagagcagaccttgagtacgtgcgtctctgcacgtatgagagcagaccttgagtacgtgcgtctctgcacgtatgagagcatattaaggtgacgcgtgtggcctcgaacaccgagcgaccctgcagcgacccgcttaaaaggcgcgcc

SEQ ID NO: 15 - DNA, 351 bp, ARTIFICIAL SEQUENCE
  SYNTHETIC PROMOTER
ttccgggaaagggtgggcaagtttccgggaaagcagtaggtacagccttccgggaaagggtgggcaagtttccgggaaagcagtaggtacagccgaccttgagtacgtgcgtctctgcacgtatgagagcagaccttgagtacgtgcgtctctgcacgtatgagagcagggaatttccggggactttccgggaatttccggggactttccgggaatttccagagcagggaatttccggggactttccgggaatttccggggactttccgggaatttccagagcatattaaggtgacgcgtgtggcctcgaacaccgagcgaccctgcagcgacccgcttaaaaggcgcgcc

SEQ ID NO: 16 - DNA, 341 bp, ARTIFICIAL SEQUENCE
  SYNTHETIC PROMOTER
ttccgggaaagggtgggcaagtttccgggaaagcagtaggtacagccttccgggaaagggtgggcaagtttccgggaaagagcagggaatttccggggactttccgggaatttccggggactttccgggaatttccagagcagggaatttccggggactttccgggaatttccggggactttccgggaatttccagagcagaccttgagtacgtgcgtctctgcacgtatgagagcagaccttgagtacgtgcgtctctgcacgtatgagagcatattaaggtgacgcgtgtggcctcgaacaccgagcgaccctgcagcgacccgcttaaaaggcgcgcc

SEQ ID NO: 17 - DNA, 341 bp, ARTIFICIAL SEQUENCE
  SYNTHETIC PROMOTER
gaccttgagtacgtgcgtctctgcacgtatgagagcagaccttgagtacgtgcgtctctgcacgtatgagagcattccgggaaagggtgggcaagtttccgggaaagcagtaggtacagccttccgggaaagggtgggcaagtttccgggaaagagcagggaatttccggggactttccgggaatttccggggactttccgggaatttccagagcagggaatttccggggactttccgggaatttccggggactttccgggaatttccagagcatattaaggtgacgcgtgtggcctcgaacaccgagcgaccctgcagcgacccgcttaaaaggcgcgcc

SEQ ID NO: 18 - DNA, 246 bp, ARTIFICIAL SEQUENCE
  SYNTHETIC PROMOTER
ttccgggaaagggtgggcaagtttccgggaaagcagtaggtacagccgaccttgagtacgtgcgtctctgcacgtatgagagcagaccttgagtacgtgcgtctctgcacgtatgagagcagggaatttccggggactttccgggaatttccggggactttccgggaatttccagagcatattaaggtgacgcgtgtggcctcgaacaccgagcgaccctgcagcgacccgcttaaaaggcgcgcc

SEQ ID NO: 19 - DNA, 169 bp, ARTIFICIAL SEQUENCE
  SYNTHETIC PROMOTER
ttccgggaaagggtgggcaagtttccgggaacccgaccttgagtacgtgcgtctctgcacgtatgtacagcgcttcctgacagtgacgcgagccgagagcatattaaggtgacgcgtgtggcctcgaacaccgagcgaccctgcagcgacccgcttaaaagcggccgcc

SEQ ID NO: 20 - DNA, 169 bp, ARTIFICIAL SEQUENCE
  SYNTHETIC PROMOTER
ttccgggaaagggtgggcaagtttccgggaacccgggaatttccggggactttccgggaatttcctacagcgcttcctgacagtgacgcgagccgagagcatattaaggtgacgcgtgtggcctcgaacaccgagcgaccctgcagcgacccgcttaaaagcggccgcc

SEQ ID NO: 21 - DNA, 174 bp, ARTIFICIAL SEQUENCE
  SYNTHETIC PROMOTER
ttccgggaaagggtgggcaagtttccgggaacccgggaatttccggggactttccgggaatttcctacagaccttgagtacgtgcgtctctgcacgtatgagagcatattaaggtgacgcgtgtggcctcgaacaccgagcgaccctgcagcgacccgcttaaaagcggccgcc

SEQ ID NO: 22 - DNA, 250 bp, ARTIFICIAL SEQUENCE
  SYNTHETIC PROMOTER
tacagggacagcagagatccagtttggactagcccggtcgcactagttctagaacttcccggaaatagggtgggcaagtatttccgggaaattctagagggagttcccggggactttccggggattttctctagatattaaggtgacgcgtgtggcctcgaacaccgagcgaccctgcagcgacccgcttaaaagcggccgccatgggccgccatggcctcctccgaggacgtcatcaaggagttcatgc

SEQ ID NO: 23 - DNA, 250 bp, ARTIFICIAL SEQUENCE
  SYNTHETIC PROMOTER
tacagggacagcagagatccagtttggactagcccggtcgcactagttctagaacttcccggaagtagggtgggcaagtacttcccggaagttctagaggaaattttcggggactttccgggggttctctctagatattaaggtgacgcgtgtggcctcgaacaccgagcgaccctgcagcgacccgcttaaaagcggccgccatgggccgccatggcctcctccgaggacgtcatcaaggagttcatgc

SEQ ID NO: 24 - DNA, 250 bp, ARTIFICIAL SEQUENCE
  SYNTHETIC PROMOTER
tacagggacagcagagatccagtttggactagcccggtcgcactagttctagaacttcccggaagtagggtgggcaagtacttccgggaaattctagagggagttctcggggactttccgggaattttctctagatattaaggtgacgcgtgtggcctcgaacaccgagcgaccctgcagcgacccgcttaaaagcggccgccatgggccgccatggcctcctccgaggacgtcatcaaggagttcatgc

SEQ ID NO: 25 - DNA, 250 bp, ARTIFICIAL SEQUENCE
  SYNTHETIC PROMOTER
tacagggacagcagagatccagtttggactagcccggtcgcactagttctagaacttcccggaagtagggtgggcaagtatttcccggaagttctagaggaagttctcggggactttccggagattctctctagatattaaggtgacgcgtgtggcctcgaacaccgagcgaccctgcagcgacccgcttaaaagcggccgccatgggccgccatggcctcctccgaggacgtcatcaaggagttcatgc

SEQ ID NO: 26 - DNA, 250 bp, ARTIFICIAL SEQUENCE
  SYNTHETIC PROMOTER
tacagggacagcagagatccagtttggactagcccggtcgcactagttctagaacttccgggaaatagggtgggcaagtacttccgggaaattctagaggggatttccggggactttccggaggttctctctagatattaaggtgacgcgtgtggcctcgaacaccgagcgaccctgcagcgacccgcttaaaagcggccgccatgggccgccatggcctcctccgaggacgtcatcaaggagttcatgc

SEQ ID NO: 27 - DNA, 250 bp, ARTIFICIAL SEQUENCE
  SYNTHETIC PROMOTER
tacagggacagcagagatccagtttggactagcccggtcgcactagttctagaacttccgggaaatagggtgggcaagtacttccgggaagttctagaggaggttttcggggactttccggaggtttcctctagatattaaggtgacgcgtgtggcctcgaacaccgagcgaccctgcagcgacccgcttaaaagcggccgccatgggccgccatggcctcctccgaggacgtcatcaaggagttcatgc

SEQ ID NO: 28 - DNA, 250 bp, ARTIFICIAL SEQUENCE
  SYNTHETIC PROMOTER
tacagggacagcagagatccagtttggactagcccggtcgcactagttctagaacttccgggaagtagggtgggcaagtatttcccggaagttctagagggggttttcggggactttccggaggtttcctctagatattaaggtgacgcgtgtggcctcgaacaccgagcgaccctgcagcgacccgcttaaaagcggccgccatgggccgccatggcctcctccgaggacgtcatcaaggagttcatgc

SEQ ID NO: 29 - DNA, 250 bp, ARTIFICIAL SEQUENCE
  SYNTHETIC PROMOTER
tacagggacagcagagatccagtttggactagcccggtcgcactagttctagaacttccgggaagtagggtgggcaagtatttccgggaaattctagagggagttctcggggactttccggggattttctctagatattaaggtgacgcgtgtggcctcgaacaccgagcgaccctgcagcgacccgcttaaaagcggccgccatgggccgccatggcctcctccgaggacgtcatcaaggagttcatgc

SEQ ID NO: 30 - DNA, 250 bp, ARTIFICIAL SEQUENCE
  SYNTHETIC PROMOTER
tacagggacagcagagatccagtttggactagcccggtcgcactagttctagaatttcccggaaatagggtgggcaagtacttccgggaaattctagagggggtttccggggactttccgggggttttctctagatattaaggtgacgcgtgtggcctcgaacaccgagcgaccctgcagcgacccgcttaaaagcggccgccatgggccgccatggcctcctccgaggacgtcatcaaggagttcatgc

SEQ ID NO: 31 - DNA, 250 bp, ARTIFICIAL SEQUENCE
  SYNTHETIC PROMOTER
tacagggacagcagagatccagtttggactagcccggtcgcactagttctagaatttcccggaaatagggtgggcaagtatttcccggaaattctagagggggttttcggggactttccgggaattttctctagatattaaggtgacgcgtgtggcctcgaacaccgagcgaccctgcagcgacccgcttaaaagcggccgccatgggccgccatggcctcctccgaggacgtcatcaaggagttcatgc

SEQ ID NO: 32 - DNA, 250 bp, ARTIFICIAL SEQUENCE
  SYNTHETIC PROMOTER
tacagggacagcagagatccagtttggactagcccggtcgcactagttctagaatttcccggaaatagggtgggcaagtatttccgggaaattctagaggaggttctcggggactttccgggagttttctctagatattaaggtgacgcgtgtggcctcgaacaccgagcgaccctgcagcgacccgcttaaaagcggccgccatgggccgccatggcctcctccgaggacgtcatcaaggagttcatgc

SEQ ID NO: 33 - DNA, 250 bp, ARTIFICIAL SEQUENCE
  SYNTHETIC PROMOTER
tacagggacagcagagatccagtttggactagcccggtcgcactagttctagaatttcccggaaatagggtgggcaagtatttccgggaaattctagaggaggttttcggggactttccgggagtttcctctagatattaaggtgacgcgtgtggcctcgaacaccgagcgaccctgcagcgacccgcttaaaagcggccgccatgggccgccatggcctcctccgaggacgtcatcaaggagttcatgc

SEQ ID NO: 34 - DNA, 250 bp, ARTIFICIAL SEQUENCE
  SYNTHETIC PROMOTER
tacagggacagcagagatccagtttggactagcccggtcgcactagttctagaatttcccggaaatagggtgggcaagtatttccgggaagttctagaggaagttttcggggactttccgggaattttctctagatattaaggtgacgcgtgtggcctcgaacaccgagcgaccctgcagcgacccgcttaaaagcggccgccatgggccgccatggcctcctccgaggacgtcatcaaggagttcatgc

SEQ ID NO: 35 - DNA, 250 bp, ARTIFICIAL SEQUENCE
  SYNTHETIC PROMOTER
tacagggacagcagagatccagtttggactagcccggtcgcactagttctagaatttccgggaaatagggtgggcaagtatttcccggaagttctagaggagattctcggggactttccgggggttctctctagatattaaggtgacgcgtgtggcctcgaacaccgagcgaccctgcagcgacccgcttaaaagcggccgccatgggccgccatggcctcctccgaggacgtcatcaaggagttcatgc

SEQ ID NO: 36 - DNA, 250 bp, ARTIFICIAL SEQUENCE
  SYNTHETIC PROMOTER
tacagggacagcagagatccagtttggactagcccggtcgcactagttctagaatttccgggaagtagggtgggcaagtacttccgggaaattctagagggggtttccggggactttccggagattctctctagatattaaggtgacgcgtgtggcctcgaacaccgagcgaccctgcagcgacccgcttaaaagcggccgccatgggccgccatggcctcctccgaggacgtcatcaaggagttcatgc

SEQ ID NO: 37 - DNA, 249 bp, ARTIFICIAL SEQUENCE
  SYNTHETIC PROMOTER
tacagggacagcagagatccagtttggactagcccggtcgcactagttctagaatttccgggaaatagggtgggcaagtatttcccggaagttctagagggggttttcggggactttccggaaattttctctagatattaaggtgacgcgtgtggcctcgaacaccgagcgaccctgcagcgacccgcttaaaagcggccgccatgggccccatggcctcctccgaggacgtcatcaaggagttcatgc

SEQ ID NO: 38 - DNA, 249 bp, ARTIFICIAL SEQUENCE
  SYNTHETIC PROMOTER
tacagggacagcagagatccagtttggactagcccggtcgcactagttctagaacttcccggaaatagggtgggcaagtatttcccggaagttctagaggaggttttcggggactttccgggattccctctagatattaaggtgacgcgtgtggcctcgaacaccgagcgaccctgcagcgacccgcttaaaagcggccgccatgggccgccatggcctcctccgaggacgtcatcaaggagttcatgc

SEQ ID NO: 39 - DNA, 243 bp, ARTIFICIAL SEQUENCE
  SYNTHETIC PROMOTER
tacagggacagcagagatccagtttggactagcccggtcgcactagttctagttccgggaagtgggtgggcaatatttcccggaagtttagaggaagttttcggggacttccggaaattccctctagatattaaggtgacgcgtgtggcctcgaacaccgagcgaccctgcagcgacccgcttaaaagcggccgccatgggccgccatggcctcctccgaggacgtcatcaaggagttcatgc

SEQ ID NO: 40 - DNA, 200 bp, ARTIFICIAL SEQUENCE
  SYNTHETIC PROMOTER
tacagggacagcagagatccagtttggactagcccggtcgcactagttctagaacttctcggaaatagggtgggcaagtactgtggcctcgaacaccgagcgaccctgcagcgacccgcttaaaagcggccgccatgggccgccatggcctcctccgaggacgtcatcaaggagttcatgcagaccaagtctctgctacc

SEQ ID NO: 41 - DNA, 250 bp, ARTIFICIAL SEQUENCE
  SYNTHETIC PROMOTER
tacagggacagcagagatccagtttggactagcccggtcgcactagttctagaayttccsggaartagggtgggcaagtayttccsggaarttctagaggrrrttyycggggactttccggrrrttyyctctagatattaaggtgacgcgtgtggcctcgaacaccgagcgaccctgcagcgacccgcttaaaagcggccgccatgggccgccatggcctcctccgaggacgtcatcaaggagttcatgc

SEQ ID NO: 42 - DNA, 50 bp, ARTIFICAL SEQUENCE
acgtggctggagtcacagtcctcttacgtggctggagtcacagtcctctt

SEQ ID NO: 43 - DNA, 50 bp, ARTIFICAL SEQUENCE
rcgtgsctggagtmacagtcctcttrcgtgsctggagtmacagtcctctt

SEQ ID NO: 44 - DNA, 39 bp, ARTIFICAL SEQUENCE
acttccsggaartagggtgggcaagtacttccsggaart

SEQ ID NO: 45 - DNA, 30 bp, ARTIFICAL SEQUENCE
gggggtttycggggactttccggrrrtttt

SEQ ID NO: 46 - DNA, 255 bp, ARTIFICAL SEQUENCE
acgtggctggagtcacagtcctcttacgtggctggagtcacagtcctcttactagttctagaacttcccggaagtagggtgggcaagtacttcccggaagttctagaggaaattttcggggactttccgggggttctctctagatattaaggtgacgcgtgtggcctcgaacaccgagcgaccctgcagcgacccgcttaaaagcggccgccatgggccgccatggcctcctccgaggacgtcatcaaggagttc

SEQ ID NO: 47 - DNA, 255 bp, ARTIFICAL SEQUENCE
aagaggactgtgactccagccacgtaagaggactgtgactccagccacgtactagttctagaacttcccggaagtagggtgggcaagtacttcccggaagttctagaggaaattttcggggactttccgggggttctctctagatattaaggtgacgcgtgtggcctcgaacaccgagcgaccctgcagcgacccgcttaaaagcggccgccatgggccgccatggcctcctccgaggacgtcatcaaggagttc